European Patent Specification EP 3 841 218 B1, published June 26, 2024. Title: Nucleic acid based detection methods. Applicant: Aptamer Diagnostics Limited. The sequence listing filed with the application follows.

SEQUENCE LISTING (4 sequences)

SEQ ID NO: 1 - DNA, 100 bp, Artificial Sequence
  Aptamer A
atccacgctctttttctccccccgctatgtgaggctcgatcgttcggtgtgtttttaaagggtacagatcctgggcggggggcattgagggtgacatagg

SEQ ID NO: 2 - DNA, 12 bp, Artificial Sequence
  Immobilization oligonucleotide
gatcgagcctca

SEQ ID NO: 3 - DNA, 19 bp, Artificial Sequence
  capture oligonucleotide (revFOR)
ggagaaaaagagcgtggat

SEQ ID NO: 4 - DNA, 19 bp, Artificial Sequence
  capture oligonucleotide (REV)
cctatgtcaccctcaatgc